European Patent Application EP 4 442 280 A1, published October 9, 2024. Title: Establishment of a method of treating and diagnosing allergic disease by regulation of immunogloblin-binding protein. Applicant: 地方独立行政法人神奈川県立産業技術総合研究所. The sequence listing filed with the application follows.

SEQUENCE LISTING (16 sequences)

SEQ ID NO: 1 - protein, 607 aa, Ruminococcus gnavus
MYRKKLMRACLTGLMVVTVATANVAPVFAAEAPAEETVQEPGAGAVGADVTVKFVDERGNVIDEKNLSFDEGIYNYEMLDQYLPAGYERKSMGDFHALQGAVIEVRVMQKAPVEEVQNVKINYYDEAAGKQVAEVPVQVSSNASVVDMAILTRYLPAGYTLEGSDCEIRGGYVYVSVAPAEEVQNVKINYYDEAAKKQVAEVPVQVSIDTSYVDMAILTRYLPEGYTLEGSDCIIRDGYVYVSVAPAEEVQNVKINYYDEAAKKQVAEVPVQVSIDTSYVDMAILTRYLPKGYTIEGTDCIIRDGYVYVSVAPAEEVQNVKINYYDEDAEKQVAEVPVQVSIDTSCVNMAILTRYMPEGYALVSSDCIIRDGYVYVSVKKDVEIREAVLHITFETPNGEVVTTETVTAEGADGEDAVFRLGVDFNLPTGYKLSNDRDQVTEITIPFGSTGGHTMVVEKGDLSSIVKIQFVDAENNDEVVAGGDYFVDGDGDGIFHTREITEWVPEGYELQEVGDFQVELYKETPLQLSVTKIKEDKPETPDPEEPNKPEDPDKEDTNNKDDKKEDTKKEDKKKNSPKTGDETSAAAAALPAGVSLAAILAVLVKKFK

SEQ ID NO: 2 - protein, 625 aa, Ruminococcus gnavus
MYRKKLMRVCLTGVMVVSIATANVAPVFAAEPVEKVETESDSWDSISGEINFRDTDNNESIFVQFNNEKVEDYRWGDDPKDTYEVLPAETVKKYLPEGYELVEGIYSVAGGETQDSYFVYAEVKKVLVEETQDVKINYYDEAAGKQVAEVPVQVSIDTSCVNMAILTRYLPEGYTLEGSDCIIRDGYVYVSVAPAEEVQNVKINYYDEAAKKQVAEVPVQVSIDTSCVNMAILTRYLPEGYTLEGSDCIIRDGYVYVSVAPAEEVQNVKINYYDEAAKKQVAEVPVQVSIDTSCVNMAILTRYLPEGYTIEGTDCIIRDGYVYVSVAPAEEVQNVKINYYDEDAEKQVAEVPVQVSIDTSCVNMAILTRYMPEGYALVSSDCIIRDGYVYVSVKKDVEIREAVLHITFETPNGEVVTTETVTAEGADGEDAVFRLGVDFNLPTGYKLSNDRDQVTEITIPFGSTGGHTMVVEKGDLSSIVKIQFVDAENNDEVVAGGDYFVDGDGDGIFHTREITEWVPEGYELQEVGDFQVELYKETPLQLSVTKIKEDKPETPDPEEPNKPEKPEDPDKEDTNNKDDKKEDTKKEDKKKNSPKTGDETSAAAAALPAGVSLAAILAVLVKKFK

SEQ ID NO: 3 - DNA, 25 bp, synthetic construct
  misc_feature 1..25: note = ibpA-F
  source 1..25: mol_type = other DNA
tgcttaacaggacttatggttgtga

SEQ ID NO: 4 - DNA, 22 bp, synthetic construct
  misc_feature 1..22: note = ibpA-R
  source 1..22: mol_type = other DNA
tgtaacgcatggaaatctccca

SEQ ID NO: 5 - DNA, 26 bp, synthetic construct
  misc_feature 1..26: note = ibpB-F
  source 1..26: mol_type = other DNA
acaggtatcaattgatacatcatgtg

SEQ ID NO: 6 - DNA, 28 bp, synthetic construct
  misc_feature 1..28: note = ibpB-F
  source 1..28: mol_type = other DNA
tctctttcttacgggtcttagtatacca

SEQ ID NO: 7 - DNA, 49 bp, synthetic construct
  misc_feature 1..49: note = His6-ibpA-F
  source 1..49: mol_type = other DNA
acatatgcatcatcatcatcatcacgtggctgaagcaccagcagaagag

SEQ ID NO: 8 - DNA, 49 bp, synthetic construct
  misc_feature 1..49: note = ibpA-,C200,B-R
  source 1..49: mol_type = other DNA
tgttagcagccggatctcaatttttcttcttatcttctttcttagtatc

SEQ ID NO: 9 - DNA, 49 bp, synthetic construct
  misc_feature 1..49: note = His6-ibpB-F
  source 1..49: mol_type = other DNA
tatacatatgcatcatcatcatcatcacgtggcagagccagtggaaaag

SEQ ID NO: 10 - DNA, 39 bp, synthetic construct
  misc_feature 1..39: note = ibpA-N100-R
  source 1..39: mol_type = other DNA
ttgttagcagccggatctcatccagctgcttcatcgtag

SEQ ID NO: 11 - DNA, 43 bp, synthetic construct
  misc_feature 1..43: note = ibpA-N200-R
  source 1..43: mol_type = other DNA
ttgttagcagccggatctcattcaagtgtatatccttctggca

SEQ ID NO: 12 - DNA, 44 bp, synthetic construct
  misc_feature 1..44: note = ibpA-CR,N349, B-N364-R
  source 1..44: mol_type = other DNA
ttgttagcagccggatctcatacagaaacatatacgtatccatc

SEQ ID NO: 13 - DNA, 41 bp, synthetic construct
  misc_feature 1..41: note = ibpA-N400-R
  source 1..41: mol_type = other DNA
ttgttagcagccggatctcatcctgttggaagattgaagtc

SEQ ID NO: 14 - DNA, 44 bp, synthetic construct
  misc_feature 1..44: note = ibpA-CR-F
  source 1..44: mol_type = other DNA
atcatcatcatcatcacgtgaaagcacctgtagaagaagtacag

SEQ ID NO: 15 - DNA, 44 bp, synthetic construct
  misc_feature 1..44: note = ibpA-C200-F
  source 1..44: mol_type = other DNA
tcatcatcatcatcacgtgtatgtttctgtaaagaaagatgtag

SEQ ID NO: 16 - DNA, 44 bp, synthetic construct
  misc_feature 1..44: note = ibpB-N200-R
  source 1..44: mol_type = other DNA
ttgttagcagccggatctcaatttacacacgatgtatcaattga